European Patent Application EP 4 631 974 A1, published October 15, 2025. Title: Antibody specifically binding to RSV. Applicant: Najing Vazyme Biotech Co., Ltd. Application CN PCT/CN2023/137389, filed December 8, 2023. The sequence listing filed with the application follows.

SEQUENCE LISTING (250 sequences)

SEQ ID NO: 1 - protein, 8 aa, Synthetic construct
GFAFRSHA

SEQ ID NO: 2 - protein, 8 aa, Synthetic construct
ISYDGGHT

SEQ ID NO: 3 - protein, 19 aa, Synthetic construct
ARSEGSYRSWPGYFYYMDV

SEQ ID NO: 4 - protein, 9 aa, Synthetic construct
SSDVGGYYY

SEQ ID NO: 5 - skipped

SEQ ID NO: 6 - protein, 11 aa, Synthetic construct
NSYSSSTIPYV

SEQ ID NO: 7 - protein, 126 aa, Synthetic construct
QEQLMESGGDVVRPGTSLTLSCKASGFAFRSHALHWVRQAPGKGLEWVSVISYDGGHTNSADSLEGRFTVSRDNSKNILYLQMNSLRTEDTAVYFCARSEGSYRSWPGYFYYMDVWGNGTTVTVSS

SEQ ID NO: 8 - protein, 111 aa, Synthetic construct
QSALTQPASVSGSPGQSITISCIGTSSDVGGYYYVSWYQQHPGRAPKLIIFDVTDRPSGVSSRFSGSQSGNTASLTISGLQPEDEADYYCNSYSSSTIPYVFGSGTKVTVL

SEQ ID NO: 9 - protein, 8 aa, Synthetic construct
GFTFKSHA

SEQ ID NO: 10 - protein, 8 aa, Synthetic construct
VPYDGATN

SEQ ID NO: 11 - protein, 20 aa, Synthetic construct
ARGATSGSYSFLGYNYYMDV

SEQ ID NO: 12 - protein, 9 aa, Synthetic construct
SSDVGAYTY

SEQ ID NO: 13 - skipped

SEQ ID NO: 14 - protein, 10 aa, Synthetic construct
SSYTDRNTLV

SEQ ID NO: 15 - protein, 127 aa, Synthetic construct
QVHLVESGGNVVHPGTSLSLSCAGSGFTFKSHAIHWVRQAPGRGLEWVAFVPYDGATNYYADSLKGRFTVSRDNSRNTVSLHMNRLEGQDTAVYFCARGATSGSYSFLGYNYYMDVWGRGTTVTVSS

SEQ ID NO: 16 - protein, 110 aa, Synthetic construct
QSALTQPASVSGSPGQSITISCTGTSSDVGAYTYVSWYQQLPGKAPKLLLFDVTDRPSGVAHRFSGSKSGNTASLTISGLQAEDEAEYYCSSYTDRNTLVFGGGTKLTVL

SEQ ID NO: 17 - protein, 8 aa, Synthetic construct
GFTLKNYA

SEQ ID NO: 18 - protein, 8 aa, Synthetic construct
TAYDGFTS

SEQ ID NO: 19 - protein, 19 aa, Synthetic construct
ARGGEGAFSWLGYLQYMDV

SEQ ID NO: 20 - protein, 9 aa, Synthetic construct
SNDIGSYTY

SEQ ID NO: 21 - skipped

SEQ ID NO: 22 - protein, 10 aa, Synthetic construct
NSYTINNTLK

SEQ ID NO: 23 - protein, 126 aa, Synthetic construct
QVQLEESGGGVVQPGRSLTLSCAASGFTLKNYAIHWVRQAPGKGLEWVAVTAYDGFTSYYADSVKSRITISRDNSKNTAYLHLNNVRDDDAAFYYCARGGEGAFSWLGYLQYMDVWGRGTTVAVSS

SEQ ID NO: 24 - protein, 110 aa, Synthetic construct
QSTLTQPASASGSPGQSITISCTGTSNDIGSYTYVSWYQHHPGKAPKLMIYDVNERPSGISHRFSGSKSGNTASLTISGLQPEDEADYYCNSYTINNTLKFGGGTRLTVL

SEQ ID NO: 25 - protein, 8 aa, Synthetic construct
GFALKSYA

SEQ ID NO: 26 - protein, 8 aa, Synthetic construct
VPYDAVTN

SEQ ID NO: 27 - protein, 20 aa, Synthetic construct
ARGATSGSYSFLGYNYYMDV

SEQ ID NO: 28 - protein, 9 aa, Synthetic construct
SSDVGAYTY

SEQ ID NO: 29 - skipped

SEQ ID NO: 30 - protein, 10 aa, Synthetic construct
SSYTDRNTIV

SEQ ID NO: 31 - protein, 127 aa, Synthetic construct
QVQLLESGGNVVQPGRSLSLSCVASGFALKSYAVHWVRQAPGKGLEWVAFVPYDAVTNYYADSVKGRFTVSRDISKNTVNLHMNRLMGEDTAVYFCARGATSGSYSFLGYNYYMDVWGRGTAVTVSS

SEQ ID NO: 32 - protein, 110 aa, Synthetic construct
QSALTQPASVSGSPGQPITISCTGTSSDVGAYTYVSWYQHHPGKAPKLILFDVTDRPSGVSHRFSGSKSGNTASLTISGLQSEDEAEYYCSSYTDRNTIVFGGGTTLTVL

SEQ ID NO: 33 - protein, 8 aa, Synthetic construct
GFTFRHYA

SEQ ID NO: 34 - protein, 8 aa, Synthetic construct
LPYDGSTK

SEQ ID NO: 35 - protein, 20 aa, Synthetic construct
ARSTYSYEYSFLGYFYYMDV

SEQ ID NO: 36 - protein, 9 aa, Synthetic construct
SRDVGAYTY

SEQ ID NO: 37 - skipped

SEQ ID NO: 38 - protein, 10 aa, Synthetic construct
SSYTDSNTVV

SEQ ID NO: 39 - protein, 127 aa, Synthetic construct
QVQLVESGGGVVLPGTSLTLSCAASGFTFRHYAIHWVRQTPGGGLEWVAALPYDGSTKYFAESVKDRFTIYRDNSQAAAFLHMSSLTPGDTALYYCARSTYSYEYSFLGYFYYMDVWGRGTSVTVSS

SEQ ID NO: 40 - protein, 110 aa, Synthetic construct
QSALTQPASVSGSPGQSISISCTGTSRDVGAYTYISWSQQHTGQAPKLLIYDVSERPSGVSDRFSGSKTGDTASLAISGLQAEDEAVYYCSSYTDSNTVVFGGGTKVTVL

SEQ ID NO: 41 - protein, 8 aa, Synthetic construct
GFAFRSHA

SEQ ID NO: 42 - protein, 8 aa, Synthetic construct
ISYDGGHT

SEQ ID NO: 43 - protein, 19 aa, Synthetic construct
ARSEGSYRSWPGYFYYMDV

SEQ ID NO: 44 - protein, 9 aa, Synthetic construct
SSDVGGYYY

SEQ ID NO: 45 - skipped

SEQ ID NO: 46 - protein, 11 aa, Synthetic construct
NSYSSSTTPYV

SEQ ID NO: 47 - protein, 126 aa, Synthetic construct
QVQLVESGGDVVRPGTSLRLSCAASGFAFRSHALHWVRQAPGKGLEWVSVISYDGGHTNSADSVKGRFTVSRDNSKNILFLQMNSLRIEDTAVYFCARSEGSYRSWPGYFYYMDVWGNGTTVTVSS

SEQ ID NO: 48 - protein, 111 aa, Synthetic construct
QSALTQPASVSGSPGQSITISCIGTSSDVGGYYYVSWYQQHPGKAPKLIIFDVSDRPSGVSSRFSGSQSGNTASLTISGLQAEDEADYYCNSYSSSTTPYVFGSGTKVTVL

SEQ ID NO: 49 - protein, 10 aa, Synthetic construct
GFSLSTRGMC

SEQ ID NO: 50 - protein, 7 aa, Synthetic construct
IDWDDDK

SEQ ID NO: 51 - protein, 18 aa, Synthetic construct
ARIRCYDYVWGDDEVFDI

SEQ ID NO: 52 - protein, 8 aa, Synthetic construct
TSNIGSNN

SEQ ID NO: 53 - skipped

SEQ ID NO: 54 - protein, 11 aa, Synthetic construct
AAWDDSLNGLL

SEQ ID NO: 55 - protein, 126 aa, Synthetic construct
QVTLRQSGPALVKPTQTLTLTCTFSGFSLSTRGMCVNWIRQPPGKALEWLARIDWDDDKYYTTSLKTRLTISKDTAKNHVVLSMTNMDPVDTATYYCARIRCYDYVWGDDEVFDIWGQGTMVSVSS

SEQ ID NO: 56 - protein, 110 aa, Synthetic construct
QSVLTQPPSASGTPGQSVTISCSGSTSNIGSNNVNWYQQLPGAAPKLVIHTNDQRPSRVPDRFSGSTSGTSASLAISGLQSEDEADYYCAAWDDSLNGLLFGGGTKLTVL

SEQ ID NO: 57 - protein, 8 aa, Synthetic construct
GFSFKMHA

SEQ ID NO: 58 - protein, 8 aa, Synthetic construct
IPYDGSSQ

SEQ ID NO: 59 - protein, 20 aa, Synthetic construct
ARGGEEGAWSWIGYNSYMDV

SEQ ID NO: 60 - protein, 9 aa, Synthetic construct
SSDVGGYDY

SEQ ID NO: 61 - skipped

SEQ ID NO: 62 - protein, 10 aa, Synthetic construct
SSYTSSNTLI

SEQ ID NO: 63 - protein, 127 aa, Synthetic construct
QVQVVESGGGVVEPGGSLSLSCAASGFSFKMHAMHWVRQAPGKGLEWVAFIPYDGSSQYYADSVKGRFTIYRDNFKNTLYLQMNSLRVEDTSLYYCARGGEEGAWSWIGYNSYMDVWGRGTAVTVSS

SEQ ID NO: 64 - protein, 110 aa, Synthetic construct
QSALTQPASVSGSPGQSITISCSGTSSDVGGYDYVCWYQKHPGESPRLIIYDVSRRPSGVSNRFSGSKSGNTASLTISGLQAEDEADYSCSSYTSSNTLIFGGGTKLTVL

SEQ ID NO: 65 - protein, 8 aa, Synthetic construct
GFTFKSYG

SEQ ID NO: 66 - protein, 8 aa, Synthetic construct
LSYDGFSG

SEQ ID NO: 67 - protein, 20 aa, Synthetic construct
ARGGDGEIFSWIGYFYYMDV

SEQ ID NO: 68 - protein, 9 aa, Synthetic construct
TNDVGGYDY

SEQ ID NO: 69 - skipped

SEQ ID NO: 70 - protein, 10 aa, Synthetic construct
SSYTITNTLK

SEQ ID NO: 71 - protein, 127 aa, Synthetic construct
QVQLVESGGGLVQPGDSLRLSCAASGFTFKSYGLHWVRQAPGKGLEWVAGLSYDGFSGYYADSVKGRFTVSRDNSKNTLYLHINSLRSEDTSIYYCARGGDGEIFSWIGYFYYMDVWGKGTTVTVFS

SEQ ID NO: 72 - protein, 110 aa, Synthetic construct
QSALTQPASVSGSPGQSITISCSGTTNDVGGYDYVSWYQHHPGKAPKLLIYDVSQRPSGVSSRFSGSKSGNTASLTISGLQTDDEAHYYCSSYTITNTLKFGGGTTLTVL

SEQ ID NO: 73 - protein, 8 aa, Synthetic construct
GFTFKNFA

SEQ ID NO: 74 - protein, 8 aa, Synthetic construct
VSYDGTSK

SEQ ID NO: 75 - protein, 22 aa, Synthetic construct
ARVESSGSGHYSYLGYFYCMDV

SEQ ID NO: 76 - protein, 9 aa, Synthetic construct
RNDVGGYEY

SEQ ID NO: 77 - skipped

SEQ ID NO: 78 - protein, 10 aa, Synthetic construct
SSYTINNTLV

SEQ ID NO: 79 - protein, 129 aa, Synthetic construct
QVQLVESGGGVVQPGRSLRLSCAASGFTFKNFAMHWVRQAPGKGLEWVAAVSYDGTSKYQADSVKGRFTISRDNSKNTLYLQMNSLRAEDTAVYYCARVESSGSGHYSYLGYFYCMDVWGKGTTVTVSS

SEQ ID NO: 80 - protein, 110 aa, Synthetic construct
QSALTQPASVSASPGQSITISCTGTRNDVGGYEYVSWYQQHPDKAPKLMIFDVSNRPSGVSNRFSGSKSGNTASLTISGLQAEDEADYYCSSYTINNTLVFGGGTKVTVL

SEQ ID NO: 81 - protein, 8 aa, Synthetic construct
GNSFTRHG

SEQ ID NO: 82 - protein, 8 aa, Synthetic construct
ISAHKSNT

SEQ ID NO: 83 - protein, 20 aa, Synthetic construct
VRDVTVVTDVGSGYDFPMDV

SEQ ID NO: 84 - protein, 8 aa, Synthetic construct
NSNIGGDY

SEQ ID NO: 85 - skipped

SEQ ID NO: 86 - protein, 11 aa, Synthetic construct
ATWDDSLNGWV

SEQ ID NO: 87 - protein, 127 aa, Synthetic construct
QVQLVQSGAEVKKPGASVRVSCGASGNSFTRHGFSWVRQAPGQGLEWIGLISAHKSNTIYAQKFQGRVTVTTDTSTSTAYMELRSLRSDDTAVYYCVRDVTVVTDVGSGYDFPMDVWGQGTTVTVSS

SEQ ID NO: 88 - protein, 110 aa, Synthetic construct
QSVLTQSPSASGTPGQRVTISCSGSNSNIGGDYVHWYQQVPGTAPRLLIYNTNQRPSGVPDRFSGSKSGTSGSLAISGLRSEDEADYYCATWDDSLNGWVFGGGTKLTVL

SEQ ID NO: 89 - protein, 8 aa, Synthetic construct
GGSVSDDE

SEQ ID NO: 90 - protein, 7 aa, Synthetic construct
IDRTGSS

SEQ ID NO: 91 - protein, 19 aa, Synthetic construct
ARGGLVVTDVGRGWDAFDV

SEQ ID NO: 92 - protein, 6 aa, Synthetic construct
QHINNW

SEQ ID NO: 93 - skipped

SEQ ID NO: 94 - protein, 9 aa, Synthetic construct
QQGDSFPLT

SEQ ID NO: 95 - protein, 125 aa, Synthetic construct
QLQLHQRGAGLLKPSETLSLTCDVYGGSVSDDEWTWIRQSPGKGLEWIGQIDRTGSSNYNPSLRSRVTISPDTSNNQFSMSLTSVTAADTALYFCARGGLVVTDVGRGWDAFDVWGQGTMVTVSS

SEQ ID NO: 96 - protein, 107 aa, Synthetic construct
DIQMTQSPSSVSASVGDRITITCRASQHINNWLAWYQQKPGEAPKLLIYAASTLQRGVPSRFSGSGSGTRFTLTITSLQPEDFASYFCQQGDSFPLTFGGGTKVEIK

SEQ ID NO: 97 - protein, 8 aa, Synthetic construct
GYTFTGNA

SEQ ID NO: 98 - protein, 8 aa, Synthetic construct
ISVNNGNT

SEQ ID NO: 99 - protein, 16 aa, Synthetic construct
AREVVNYGSGSLNFDS

SEQ ID NO: 100 - protein, 6 aa, Synthetic construct
KLGNDY

SEQ ID NO: 101 - skipped

SEQ ID NO: 102 - protein, 9 aa, Synthetic construct
QAWDGSTVI

SEQ ID NO: 103 - protein, 123 aa, Synthetic construct
QVQLVQSGTEVKKPGASVKISCKASGYTFTGNAINWVRQAPGQGLEWLGWISVNNGNTKYVQKFQGRVTMTTDTSTSTAYMELRSLGSDDTAVYYCAREVVNYGSGSLNFDSWGQGTLVTVSS

SEQ ID NO: 104 - protein, 106 aa, Synthetic construct
SYELTQPPSVSVSPGQTVSISCSGDKLGNDYVSWYQQKPGQSPVLVIYEDSKRPSGIPERFSGSNSGNTATLTISGTQAMDESDYYCQAWDGSTVIFGGGTKLTVL

SEQ ID NO: 105 - protein, 8 aa, Synthetic construct
EFTFSTDF

SEQ ID NO: 106 - protein, 8 aa, Synthetic construct
ITPSDGTT

SEQ ID NO: 107 - protein, 17 aa, Synthetic construct
VAYDRVTTSAGTGASDI

SEQ ID NO: 108 - protein, 11 aa, Synthetic construct
QSLLHGDGYNY

SEQ ID NO: 109 - skipped

SEQ ID NO: 110 - protein, 9 aa, Synthetic construct
MQGLQTPFT

SEQ ID NO: 111 - protein, 124 aa, Synthetic construct
QEQSVQSGAEVKKPGASVKVSCRASEFTFSTDFIHWVRQAPGQGLEWMGRITPSDGTTTYAQKFQGRVTMTRDPSTNTVYIELRRLKSEDTAVYYCVAYDRVTTSAGTGASDIWGQGTMVTVSS

SEQ ID NO: 112 - protein, 112 aa, Synthetic construct
DIVMTQSPLSLPVTPGEPASISCRSSQSLLHGDGYNYLDWYLQKPGRSPQLLIYLGSHRASGVPDRFSGSGSGTDFTLRISRVEAEDVGIYYCMQGLQTPFTFGPGTKVDIK

SEQ ID NO: 113 - protein, 8 aa, Synthetic construct
SFSVTGSY

SEQ ID NO: 114 - protein, 7 aa, Synthetic construct
IYSTGST

SEQ ID NO: 115 - protein, 19 aa, Synthetic construct
ARLGPAGGSWSWEFYGLDV

SEQ ID NO: 116 - protein, 6 aa, Synthetic construct
QGTTSY

SEQ ID NO: 117 - skipped

SEQ ID NO: 118 - protein, 9 aa, Synthetic construct
QQVNIFPYT

SEQ ID NO: 119 - protein, 125 aa, Synthetic construct
EVQVVESGGGLVQPGGSLRLSCAASSFSVTGSYMTWVRQAPGKGLESVSLIYSTGSTYYADSVKGRFVISRDDSKNILFLQMNNLRVEDTGVYFCARLGPAGGSWSWEFYGLDVWGQGTTVTVFS

SEQ ID NO: 120 - protein, 107 aa, Synthetic construct
CVQMTQSPSFLSASVGDRVTISCRASQGTTSYLAWYQQKPGKAPKLLIYGVSTLQTGVPSRFSGSGSGTDFTLTISNLQPEDFATYYCQQVNIFPYTFGPGTKVEIK

SEQ ID NO: 121 - protein, 8 aa, Synthetic construct
AYDFIDDS

SEQ ID NO: 122 - protein, 8 aa, Synthetic construct
IDPSGDTT

SEQ ID NO: 123 - protein, 17 aa, Synthetic construct
VAYERATTLAGVGASDV

SEQ ID NO: 124 - protein, 11 aa, Synthetic construct
QSLLYRDGYNY

SEQ ID NO: 125 - skipped

SEQ ID NO: 126 - protein, 9 aa, Synthetic construct
MQSLQTPFT

SEQ ID NO: 127 - protein, 124 aa, Synthetic construct
QVQLAQSGAEVRRPGTSVKVSCRSSAYDFIDDSIHWVRQAPGQGLEWMGRIDPSGDTTTYAPQFQVRITLTRDTSTSTASMELNRLTSQDTAMYYCVAYERATTLAGVGASDVWGQGTWVTVSS

SEQ ID NO: 128 - protein, 112 aa, Synthetic construct
DIVMTQSPLSLSVTPGEPASISCRSSQSLLYRDGYNYLDWYLQKPGQSPQLLLYFASYRASGVPDRFSGSGSGTDFTLTITRVEPEDVGIYYCMQSLQTPFTFGPGTKLDFK

SEQ ID NO: 129 - protein, 8 aa, Synthetic construct
GVSLSGDY

SEQ ID NO: 130 - protein, 7 aa, Synthetic construct
INHSGST

SEQ ID NO: 131 - protein, 19 aa, Synthetic construct
ARGWEYCHGTTCYSKAFDI

SEQ ID NO: 132 - protein, 6 aa, Synthetic construct
QDISNY

SEQ ID NO: 133 - skipped

SEQ ID NO: 134 - protein, 9 aa, Synthetic construct
QQFHNLPVT

SEQ ID NO: 135 - protein, 125 aa, Synthetic construct
QVQLQQWGAGLLRPSETLSLTCAVSGVSLSGDYLTWIRQTPGKGLEWIGEINHSGSTNYNPSLKSRVTISVETSKNHFSLKMRSVTAADSALYYCARGWEYCHGTTCYSKAFDIWGQGTLVTVSS

SEQ ID NO: 136 - protein, 107 aa, Synthetic construct
DIQMTQSPSSLSASVGDRVTITCQASQDISNYLIWYQQKPGRAPKLLIFDASKLEKGVPPRFSGSGSGTYFTFTISSLQPEDFATYYCQQFHNLPVTFGGGTKLETK

SEQ ID NO: 137 - protein, 8 aa, Synthetic construct
GFILSDST

SEQ ID NO: 138 - protein, 7 aa, Synthetic construct
IANGYAT

SEQ ID NO: 139 - protein, 17 aa, Synthetic construct
TSRSVVVTDVGAGRDDY

SEQ ID NO: 140 - protein, 11 aa, Synthetic construct
QSLLHRNGYNY

SEQ ID NO: 141 - skipped

SEQ ID NO: 142 - protein, 9 aa, Synthetic construct
MQDLQTPPT

SEQ ID NO: 143 - protein, 123 aa, Synthetic construct
EEQLVESGGGLVQPGGSLKLSCAASGFILSDSTVHWVRQASGRGLEWVGRIANGYATSYAASVKGRFTISTDDSGNTAYLEMNSLKTEDTAVYYCTSRSVVVTDVGAGRDDYWGQGTLVTVSS

SEQ ID NO: 144 - protein, 112 aa, Synthetic construct
DIVMTQSPLSLPVTPGEPASISCRSSQSLLHRNGYNYLDWYLQKPGQSPQLLIWLGSNRASGVPDRFSGSGSGTDFTLTISRVEAEDVGVYYCMQDLQTPPTFGGGTKVEIM

SEQ ID NO: 145 - protein, 10 aa, Synthetic construct
GFSLTTTGVA

SEQ ID NO: 146 - protein, 7 aa, Synthetic construct
IYWDDDK

SEQ ID NO: 147 - protein, 22 aa, Synthetic construct
AHFDYGDPEVVALFEYSYYMDV

SEQ ID NO: 148 - protein, 8 aa, Synthetic construct
SSNIGSNY

SEQ ID NO: 149 - skipped

SEQ ID NO: 150 - protein, 12 aa, Synthetic construct
AVWDDSVGGHWV

SEQ ID NO: 151 - protein, 130 aa, Synthetic construct
QITLKESGPTLLKPTQTLTLTCTFSGFSLTTTGVAVGWVRQPPGKALEWLALIYWDDDKRYSPSLKSRVTITKDTSKNQVLLAMTDMDPVDTATYYCAHFDYGDPEVVALFEYSYYMDVWGKGITVTVSS

SEQ ID NO: 152 - protein, 111 aa, Synthetic construct
QSVLTQPPSVSGTPGQRVTISCSGSSSNIGSNYVYWYQHLPGTAPKLLIYTNNRRPSGVPDRFSGSKSGTSASLAVSGLRSEDEADYFCAVWDDSVGGHWVFGGGTKLTVL

SEQ ID NO: 153 - protein, 8 aa, Synthetic construct
GVTRNTYA

SEQ ID NO: 154 - protein, 8 aa, Synthetic construct
TSYDGTSK

SEQ ID NO: 155 - protein, 19 aa, Synthetic construct
AKGPQGIYSYIGYFYYMDV

SEQ ID NO: 156 - protein, 9 aa, Synthetic construct
RDDVGDYDY

SEQ ID NO: 157 - skipped

SEQ ID NO: 158 - protein, 10 aa, Synthetic construct
NSYTSSNSVV

SEQ ID NO: 159 - protein, 126 aa, Synthetic construct
QVQLEESGGGVVQPGTSLRLSCSSSGVTRNTYAVHWVRQVPGKGLEWLAATSYDGTSKYYPENGHGRVSISKEYSTNMVYLEIYNLRPEDTAVYFCAKGPQGIYSYIGYFYYMDVWGKGTTVTVSS

SEQ ID NO: 160 - protein, 110 aa, Synthetic construct
QSALTQPASVSGSPGQSITLSCTGSRDDVGDYDYVSWYQHHPGKAPRLIIYDVTSRPSGVSPRFSGSKSGNTASLTISGLQADDEADYYCNSYTSSNSVVFGGGTKVTVL

SEQ ID NO: 161 - protein, 8 aa, Synthetic construct
GYTFSDYS

SEQ ID NO: 162 - protein, 8 aa, Synthetic construct
INTSGGTT

SEQ ID NO: 163 - protein, 17 aa, Synthetic construct
VAYERATTLAGAGASDI

SEQ ID NO: 164 - protein, 11 aa, Synthetic construct
QSLLHSDGYNY

SEQ ID NO: 165 - skipped

SEQ ID NO: 166 - protein, 9 aa, Synthetic construct
MQSLQTPFT

SEQ ID NO: 167 - protein, 124 aa, Synthetic construct
QERLAQSGTEVKKPGASVKVSCRALGYTFSDYSIHWVRQAPRQGLEWMGKINTSGGTTTYAQKFQARVTLTSDTSTSTASMELSSLKIEDTAVYYCVAYERATTLAGAGASDIWGQGTLVTVSS

SEQ ID NO: 168 - protein, 112 aa, Synthetic construct
DIVMTQSPLSLPVTPGEPASISCRSSQSLLHSDGYNYLDWYLQKPGQSPHLLIYLGSNRASGVPDRFSGSGSGTDFTLKITRVEPEDVGVYYCMQSLQTPFTFGPGTKVDVK

SEQ ID NO: 169 - protein, 8 aa, Synthetic construct
GYAFTDYS

SEQ ID NO: 170 - protein, 8 aa, Synthetic construct
IYPGDGHA

SEQ ID NO: 171 - protein, 17 aa, Synthetic construct
VAYERATTLAGAGASDI

SEQ ID NO: 172 - protein, 11 aa, Synthetic construct
QSLLQSDGYNY

SEQ ID NO: 173 - skipped

SEQ ID NO: 174 - protein, 9 aa, Synthetic construct
MQSLQSPFT

SEQ ID NO: 175 - protein, 124 aa, Synthetic construct
QEQLVQSGAEVKRPGTSVKVSCKASGYAFTDYSIHWVRQAPGVGLEWMGKIYPGDGHALYAQNFQGRVTLTRDTSTASVYMELRSLRSQDTAVYYCVAYERATTLAGAGASDIWGQGTMVTVSS

SEQ ID NO: 176 - protein, 112 aa, Synthetic construct
DIVMTQSPLSLPVTPGEPASISCRSSQSLLQSDGYNYMDWYLQKPGRSPQLLIYLGSHRASGVPDRFSGSGSGTDFTLRISRVKAEDVGIYYCMQSLQSPFTFGPGTKVDIK

SEQ ID NO: 177 - protein, 8 aa, Synthetic construct
EFTFSTDF

SEQ ID NO: 178 - protein, 8 aa, Synthetic construct
ITPSDGTT

SEQ ID NO: 179 - protein, 17 aa, Synthetic construct
VAYDRATTSAGAGATDI

SEQ ID NO: 180 - protein, 11 aa, Synthetic construct
QSLLHGDGYNY

SEQ ID NO: 181 - skipped

SEQ ID NO: 182 - protein, 9 aa, Synthetic construct
MQGLQTPFT

SEQ ID NO: 183 - protein, 124 aa, Synthetic construct
QEQSVQSGPEVKKPGASVKVSCRASEFTFSTDFIHWVRQAPGQGLEWMGRITPSDGTTTYAPKFQGRVAVTRDPSTKNVYIQLTRLKSEDTAVYYCVAYDRATTSAGAGATDIWGQGTLVTVSS

SEQ ID NO: 184 - protein, 112 aa, Synthetic construct
DIVMTQSPLSLPVTPGEPASISCRSSQSLLHGDGYNYLDWYLQRPGRSPQLLIYLGSHRASGVPDRFSGSGSGTDFTLRISRVEAEDVGIYYCMQGLQTPFTFGPGTKVDIK

SEQ ID NO: 185 - protein, 8 aa, Synthetic construct
GGSMSDFY

SEQ ID NO: 186 - protein, 7 aa, Synthetic construct
VHHSGKV

SEQ ID NO: 187 - protein, 19 aa, Synthetic construct
AATSAFVDSSSYSPPYFDF

SEQ ID NO: 188 - protein, 6 aa, Synthetic construct
HDITNY

SEQ ID NO: 189 - skipped

SEQ ID NO: 190 - protein, 9 aa, Synthetic construct
QQYDNLPIT

SEQ ID NO: 191 - protein, 125 aa, Synthetic construct
QVQLQQSGPGLVKPSETLSLACSVSGGSMSDFYWSWIRQSPGTGLEWIGYVHHSGKVNYNPSLKARVTMSLDTSKYLLSLNLASMTAADSAVYYCAATSAFVDSSSYSPPYFDFWGQGTLITVSS

SEQ ID NO: 192 - protein, 107 aa, Synthetic construct
DIQLTQSPSSLSASVGDRVTITCQASHDITNYLNWYQQTPGKAPRLLIYVATNLETGVPSRFSGSGSGTHFTLTISSLQPEDSATYYCQQYDNLPITFGGGTRVEIR

SEQ ID NO: 193 - protein, 106 aa, Synthetic construct
GQPKANPTVTLFPPSSEELQANKATLVCLISDFYPGAVTVAWKADGSPVKAGVETTKPSKQSNNKYAASSYLSLTPEQWKSHRSYSCQVTHEGSTVEKTVAPTECS

SEQ ID NO: 194 - protein, 107 aa, Synthetic construct
RTVAAPSVFIFPPSDEQLKSGTASVVCLLNNFYPREAKVQWKVDNALQSGNSQESVTEQDSKDSTYSLSSTLTLSKADYEKHKLYACEVTHQGLSSPVTKSFNRGEC

SEQ ID NO: 195 - protein, 106 aa, Synthetic construct
GQPKAAPSVTLFPPSSEELQANKATLVCLISDFYPGAVTVAWKADSSPVKAGVETTTPSKQSNNKYAASSYLSLTPEQWKSHKSYSCQVTHEGSTVEKTVAPTECS

SEQ ID NO: 196 - protein, 106 aa, Synthetic construct
GQPKAAPSVTLFPPSSEELQANKATLVCLISDFYPGAVTVAWKADGSPVKAGVETTTPSKQSNNKYAASSYLSLTPEQWKSHRSYSCQVTHEGSTVEKTVAPTECS

SEQ ID NO: 197 - protein, 106 aa, Synthetic construct
GQPKAAPSVTLFPPSSEELQANKATLVCLISDFYPGAVTVAWKADSSPVKAGVETTTPSKQSNNKYAASSYLSLTPEQWKSHRSYSCQVTHEGSTVEKTVAPTECS

SEQ ID NO: 198 - protein, 106 aa, Synthetic construct
GQPKAAPSVTLFPPSSEELQTNKATLVCLISDFYPGAVTVAWKADSSPVKAGVETTTPSKQSNNKYAASSYLSLTPEQWKSHRSYSCQVTHEGSTVEKTVAPTECS

SEQ ID NO: 199 - protein, 107 aa, Synthetic construct [sequence omitted]

SEQ ID NO: 200 - protein, 106 aa, Synthetic construct
RQPKAAPSVTLFPPSSEELQANEATLVCLISDFYPGAVTVAWKADSSPVKAGVETTTPSKQSNNKYAASSYLSLSPEQWKSHKSYSCQVTHEGSTVEKTVAPTECS

SEQ ID NO: 201 - protein, 330 aa, Synthetic construct
ASTKGPSVFPLAPSSKSTSGGTAALGCLVKDYFPEPVTVSWNSGALTSGVHTFPAVLQSSGLYSLSSVVTVPSSSLGTQTYICNVNHKPSNTKVDKKVEPKSCDKTHTCPPCPAPELLGGPSVFLFPPKPKDTLYITREPEVTCVVVDVSHEDPEVKFNWYVDGVEVHNAKTKPREEQYNSTYRVVSVLTVLHQDWLNGKEYKCKVSNKALPAPIEKTISKAKGQPREPQVYTLPPSRDELTKNQVSLTCLVKGFYPSDIAVEWESNGQPENNYKTTPPVLDSDGSFFLYSKLTVDKSRWQQGNVFSCSVMHEALHNHYTQKSLSLSPGK

SEQ ID NO: 202 - DNA, 378 bp, Synthetic construct
  source 1..378: mol_type = other DNA
caggagcagcttatggagtctgggggggacgtggtccggcctgggacgtccctgacactctcctgtaaagcctctggattcgccttcagaagtcacgctctccactgggtccgccaggctcccggcaaggggctagagtgggtgtctgtcatatcatatgatggaggccatacaaactctgcagactccctggagggccgattcactgtctccagagacaactccaagaacatcctgtatctgcaaatgaacagcctgagaactgaggacacggctgtctatttttgtgcgagatcggaggggtcttacaggagctggccgggttacttctactacatggatgtctggggcaacgggactacggtcaccgtctcttca

SEQ ID NO: 203 - DNA, 333 bp, Synthetic construct
  source 1..333: mol_type = other DNA
cagtctgccctgactcagcctgcctccgtgtctgggtctcctggacaatcgatcaccatctcctgcattggaaccagcagtgacgttggtggctattactatgtctcctggtaccaacaacaccccggcagagcccccaaactcatcatttttgatgtcactgatcggccctcaggggtttctagtcgcttctctggctcccagtctggcaacacggcctccctgaccatctctggcctccagcctgaggacgaggctgattattactgcaactcatattcaagtagcaccattccatatgtcttcggatctgggaccaaggtcaccgtcctg

SEQ ID NO: 204 - DNA, 381 bp, Synthetic construct
  source 1..381: mol_type = other DNA
caggtgcacttggtggagtctgggggaaacgtggtccaccctgggacgtccctgagtctctcctgtgcaggctctggatttaccttcaaatcccatgctatccactgggtccgccaggctccaggcaggggactggagtgggtggcattcgtcccatatgatggagccactaactattatgcagactccctgaagggccgattcactgtttccagagacaactccaggaacacagtcagtctacacatgaaccgcctggaaggtcaggacacggctgtctatttctgtgcgagaggggcaactagtggttcttactccttcctggggtacaactactacatggacgtctggggcagagggaccacggtcaccgtctcctca

SEQ ID NO: 205 - DNA, 330 bp, Synthetic construct
  source 1..330: mol_type = other DNA
caatctgccctgactcagcctgcctccgtgtctgggtctcctggacagtcaatcaccatctcctgcactggaacgagcagtgacgttggtgcttatacctatgtctcctggtaccaacaactcccaggcaaagcccccaaactcctactttttgatgtcactgatcggccctcaggggttgctcaccgcttctctggctccaagtctggcaacacggcctccctgaccatctctggcctccaggctgaggacgaggctgaatattactgcagctcatatacagacaggaacactcttgtgttcggcggagggaccaaattgaccgtccta

SEQ ID NO: 206 - DNA, 378 bp, Synthetic construct
  source 1..378: mol_type = other DNA
caggtgcagctggaggagtctgggggaggcgtcgtccaacctgggaggtccctgacactctcctgtgcagcctctggattcaccttgaaaaattatgccattcactgggtccgccaggctccaggcaaggggctggagtgggtggccgtcacagcatatgatggattcactagttattacgcagactctgtgaagtcccgaatcaccatctccagagacaactccaagaacacagcatatctccatctcaataacgtgagagatgacgacgcggctttctattattgtgcgagaggcggagagggtgccttcagttggttggggtatctccagtacatggacgtctgggggagagggactacggtcgccgtctcctca

SEQ ID NO: 207 - DNA, 330 bp, Synthetic construct
  source 1..330: mol_type = other DNA
caatctaccctgactcagcctgcctccgcgtctgggtctcctggacagtcgatcaccatctcctgcactggaaccagcaatgacattggttcttacacctatgtctcctggtatcaacaccacccaggcaaagcccccaaactcatgatttatgatgtcaatgaacggccctcagggatttctcatcgcttctctggctccaagtctggcaacacggcctccctgaccatctctgggctccagcctgaagacgaggctgattattattgcaactcatatacaatcaacaacactttgaaattcggcggcgggaccaggctgaccgtccta

SEQ ID NO: 208 - DNA, 381 bp, Synthetic construct
  source 1..381: mol_type = other DNA
caggtgcagttgctggagtctgggggaaacgtggtccagcctgggaggtccctgagcctctcctgtgtagcctctggatttgccttaaaatcctatgctgtccactgggtccgccaggctccaggcaaggggctggagtgggtggcattcgtcccctatgatgcagtcactaactattatgcagactccgtgaagggccgattcactgtttccagagacatctccaagaacacagtcaatctacacatgaaccgcctcatgggtgaggacacggctgtctatttctgtgcgagaggggcaactagtggttcttactccttcctggggtacaactactacatggacgtctggggccgagggaccgcggtcaccgtctcctca

SEQ ID NO: 209 - DNA, 330 bp, Synthetic construct
  source 1..330: mol_type = other DNA
caatctgccctgactcagccagcctccgtgtctgggtctcctggacagccgatcaccatctcctgcactggaacgagcagtgacgttggtgcttatacctatgtctcctggtaccaacaccacccaggcaaagcccccaaactcattctttttgatgtcactgatcggccctcaggcgtttctcatcgcttctctggctccaagtctggcaacacggcctccctgaccatctctgggctccagtctgaggacgaggctgaatattactgcagttcatatacagataggaacactattgtgttcggcggagggaccacattgaccgtccta

SEQ ID NO: 210 - DNA, 381 bp, Synthetic construct
  source 1..381: mol_type = other DNA
caagtgcagttggtggagtctgggggaggcgtggtcctgcctgggacgtccctgacactgtcttgtgcagcctctggattcaccttccgtcactatgctattcactgggtccgccagactccaggcggcggcctggagtgggtggcggctcttccatatgatggctcaactaaatacttcgcagagtcggtgaaagaccgattcaccatctacagagacaactcccaggccgcggcttttctgcacatgagcagcctgacgcctggcgacacggctctatattactgcgcgaggagcacctactcttacgaatactcctttctgggctatttttactacatggacgtctggggcagagggacctcggtcaccgtctcgtca

SEQ ID NO: 211 - DNA, 330 bp, Synthetic construct
  source 1..330: mol_type = other DNA
cagtctgccctgactcagcctgcctccgtgtctgggtctcctggacagtcgatctccatctcctgcactggaaccagtcgtgacgttggcgcttatacctacatctcctggtcccaacaacacacaggccaggcccctaaactcctaatttatgatgtctctgagcggccctcaggagtttctgatcgcttctctggctccaagactggcgacacggcctccctggccatctctgggctccaggctgaggacgaggctgtttattactgcagctcatatacagactccaacactgtggtcttcggcggagggaccaaggtgaccgtccta

SEQ ID NO: 212 - DNA, 378 bp, Synthetic construct
  source 1..378: mol_type = other DNA
caggtgcagcttgtggagtctgggggggacgtggtccggcctgggacgtccctgagactctcctgtgcagcctctggattcgccttcagaagtcatgctctccactgggtccgccaggctcccggcaaggggctggagtgggtgtctgttatatcatatgatggaggccatacaaactctgcagactccgtgaagggccgattcaccgtctccagagacaattccaagaacatcctgtttctgcaaatgaacagcctgagaattgaggacacggctgtctatttttgtgcgagatcggaggggtcttacaggagctggccgggttacttctactacatggacgtctggggcaacgggactacggtcaccgtctcttca

SEQ ID NO: 213 - DNA, 333 bp, Synthetic construct
  source 1..333: mol_type = other DNA
cagtctgccctgactcagcctgcctccgtgtctgggtctcctggacaatcgatcaccatctcctgcattggaaccagcagtgacgttggtggctattactatgtctcctggtaccaacaacacccaggcaaagcccccaaactcatcatttttgatgtcagtgatcggccctcaggggtttctagtcgcttctctggctcccagtctggcaacacggcctccctgaccatctctggcctccaggctgaggacgaggctgattattactgcaactcatattcaagtagcaccaccccatatgtcttcggatctgggaccaaggtcaccgtcctg

SEQ ID NO: 214 - DNA, 378 bp, Synthetic construct
  source 1..378: mol_type = other DNA
caggtcaccttgaggcagtctggtcctgcgctggtgaaacccacacagaccctcacactgacctgcaccttctctgggttctcactcagtactagaggaatgtgtgtgaactggatccgtcagcccccagggaaggccctggagtggcttgcacgcattgattgggatgatgataaatactacaccacatctctgaagaccaggctcaccatctctaaggacaccgccaaaaaccacgtggtcctttcaatgaccaacatggaccctgtggacacagccacatattactgtgcacggatacggtgttatgattacgtttggggggacgatgaggttttcgatatctggggccaagggacaatggtcagcgtctcctca

SEQ ID NO: 215 - DNA, 330 bp, Synthetic construct
  source 1..330: mol_type = other DNA
cagtctgtactgactcagccaccctcagcgtctgggacccccgggcagagtgtcaccatctcttgttctggaagcacctccaacatcggaagtaataatgtaaactggtaccagcagctcccaggagcggcccccaaactcgtcatccatactaatgatcagcggccctcacgggtccctgaccgattctctggctctacgtctggcacctcagcctccctggccatcagtgggctccagtctgaggatgaggctgattattactgtgcagcatgggatgacagcctgaatggtctgctgttcggcggagggaccaagctgaccgtctta

SEQ ID NO: 216 - DNA, 381 bp, Synthetic construct
  source 1..381: mol_type = other DNA
caggtacaagtggtggagtctgggggaggcgtagtggagcctggggggtccctgagcctctcctgtgcggcctctggtttcagcttcaaaatgcatgcaatgcactgggtccgccaggcgccaggcaaggggctggagtgggtggcttttataccatatgatggaagtagtcaatactacgcagactccgtgaagggccgattcaccatctacagagacaattttaagaacacactctatctgcaaatgaacagcctgagagttgaagacacgtctctgtattattgtgcgagaggaggagaagaaggcgcctggtcctggatagggtacaattcctacatggacgtctggggcagagggaccgcggtcaccgtctcctca

SEQ ID NO: 217 - DNA, 330 bp, Synthetic construct
  source 1..330: mol_type = other DNA
cagtctgccctgactcagcctgcctccgtgtctgggtctcctggacagtcgatcaccatctcctgcagtggaaccagcagtgacgttggtggttacgactatgtctgctggtaccaaaagcacccaggcgaatcgcccagactcataatttatgatgtcagtaggcggccctcaggagtttctaatcgcttctctggctccaagtctggcaacacggcctccctgaccatctctgggctccaggctgaagacgaggctgattattcctgcagttcatatacgagcagtaacactttgatattcggcggcgggaccaaactaaccgtcctg

SEQ ID NO: 218 - DNA, 381 bp, Synthetic construct
  source 1..381: mol_type = other DNA
caagtacaactggtggagtctgggggaggcctggtccagcctggggattccctgaggctctcctgtgcagcctctggattcacttttaagtcttacggtctgcactgggtccgccaggctccaggcaaggggctggagtgggtggcaggcctttcatatgatggattcagcggatactacgccgactccgtgaagggccgattcaccgtctccagagacaactccaagaacacactgtatctacacataaacagcctgagatctgaggacacgtccatatattactgtgcgagagggggcgatggggaaatcttcagttggatcggctacttctactacatggacgtctggggcaaagggaccacggtcaccgtcttctca

SEQ ID NO: 219 - DNA, 330 bp, Synthetic construct
  source 1..330: mol_type = other DNA
caatctgccctgactcagcctgcttccgtgtctgggtctcctggacagtcgatcaccatctcctgctctggaaccaccaatgacgttggtggctatgactatgtctcctggtaccaacaccacccaggcaaagcccccaaactcctgatttatgatgtctctcagcggccctcgggggtttctagtcgcttctcaggctccaagtctggcaacacggcctccctgaccatctctgggctccagactgacgacgaggctcactactactgcagctcatatacaataaccaacactttaaaatttggcggagggaccacgctgaccgtccta

SEQ ID NO: 220 - DNA, 387 bp, Synthetic construct
  source 1..387: mol_type = other DNA
caggttcagctggtggagtctgggggaggcgtggtccagcctgggaggtccctgagactctcctgtgcagcctctggattcaccttcaagaactttgctatgcactgggtccgccaggctccaggcaaggggctggagtgggtggccgctgtgtcatatgatggaaccagtaaatatcaggcagactccgtgaagggccggttcaccatctccagagacaactccaagaacacgctgtatttgcaaatgaacagcctgagagctgaggacacggctgtatattactgtgcgagagtggagagtagtggtagtggtcattactcctacctgggttacttttactgcatggacgtctggggcaaagggactacggtcaccgtctcctca

SEQ ID NO: 221 - DNA, 330 bp, Synthetic construct
  source 1..330: mol_type = other DNA
cagtctgccctgactcagcctgcctccgtgtctgcgtctcctggacagtcgatcaccatctcctgcactggaaccaggaatgacgttggtggttatgagtatgtctcatggtaccagcaacacccagacaaagcccccaaactcatgatttttgatgtcagtaatcggccctcaggggtttctaatcgcttctctggctccaagtctggcaacacggcctccctgaccatctctggactccaggctgaggacgaggctgattattactgcagctcatatacaatcaacaacactcttgtgttcggcggagggaccaaggtgaccgtccta

SEQ ID NO: 222 - DNA, 381 bp, Synthetic construct
  source 1..381: mol_type = other DNA
caggttcagttggtgcaatctggcgctgaggtgaagaagcctggggcctcagtgagggtctcctgcggggcttctggtaacagtttcaccaggcatggtttcagctgggtgcgacaggccccaggacaagggcttgagtggataggattgatcagcgctcacaaaagtaacacaatctatgcgcagaagttccagggcagagtcaccgtgaccacggacacgtccacgagtacagcctacatggagctgaggagcctgagatctgacgacacggccgtgtattactgtgtgagagacgtaaccgtggtgactgatgtcggatcggggtacgacttccctatggacgtctggggccaagggaccacagtcaccgtctcctca

SEQ ID NO: 223 - DNA, 330 bp, Synthetic construct
  source 1..330: mol_type = other DNA
cagtctgtgctgactcagtcaccctcagcgtctgggacccccgggcagagggtcaccatctcttgttctggaagcaactccaacatcggaggggattatgtacactggtaccagcaggtcccaggaacggcccccagactcctcatctataatactaatcagcggccctcaggggtccctgaccgattctctggctccaagtctggcacctcaggctccctggccatcagtggactccggtccgaggatgaggctgattattactgtgcaacatgggatgacagcctgaatggttgggtgttcggcggagggaccaagctgaccgtccta

SEQ ID NO: 224 - DNA, 375 bp, Synthetic construct
  source 1..375: mol_type = other DNA
cagctgcagctacatcagcggggcgcaggactgttgaagccttcggagaccctgtccctcacctgcgatgtctatggtgggtcggtcagtgatgacgagtggacctggatccgccagtccccagggaaggggctagagtggattggacaaatcgatcggactggaagcagcaactacaacccgtccctccggagtcgagtcaccatttcaccagacacgtccaacaatcagttttccatgagcctgacctctgtgaccgccgcggacacggctctctatttttgtgctagaggcggactggtggtgactgatgtaggacggggttgggatgcttttgatgtctggggccaagggacaatggtcaccgtctcttca

SEQ ID NO: 225 - DNA, 321 bp, Synthetic construct
  source 1..321: mol_type = other DNA
gacatccagatgacccagtctccatcttccgtgtctgcatctgtgggagacagaatcaccatcacttgtcgggcgagtcagcatattaataactggttagcctggtatcagcagaaaccaggggaagcccctaaactcctgatctatgctgcctccactttgcaaaggggggtcccatcaaggttcagcggcagtggatctgggacaagattcactctcaccatcaccagcctgcagcctgaagattttgcatcttacttttgtcaacagggtgacagtttcccgctcactttcggcggggggaccaaggtggagatcaaa

SEQ ID NO: 226 - DNA, 369 bp, Synthetic construct
  source 1..369: mol_type = other DNA
caggttcagctggtgcagtctggaactgaggtgaagaagcctggggcctcagtgaagatctcctgcaaggcttctggttacacctttaccggcaatgctatcaactgggtgcgacaggcccctggacaagggcttgagtggctgggatggatcagcgtcaacaatggtaacacaaagtatgtacagaagttccagggcagagtcaccatgaccacagacacatccacgagcacagcctacatggagctgaggagcctgggatctgacgacacggccgtgtattactgtgcgagggaggtggtcaactatggttcggggagtctaaactttgactcttggggccagggaaccctggtcaccgtctcctca

SEQ ID NO: 227 - DNA, 318 bp, Synthetic construct
  source 1..318: mol_type = other DNA
tcctacgagctgactcagccaccctcagtgtccgtgtccccaggacagacagtcagcatcagctgctctggagataaattggggaatgactatgttagttggtatcaacagaagccaggccagtcccctgtgttggtcatctatgaagattccaagcggccctcagggatccctgagcgattctctggctccaactctgggaacacagccactctgaccatcagcgggacccaggctatggatgagagtgactattactgtcaggcgtgggacggcagcactgtgattttcggcggagggaccaagctgaccgtccta

SEQ ID NO: 228 - DNA, 372 bp, Synthetic construct
  source 1..372: mol_type = other DNA
caggagcagtcggtgcagtctggggctgaggtgaagaagcctggggcctcagtgaaggtctcctgcagggcatcagaattcaccttctccaccgactttatacactgggtgcgacaagcccctggacaaggacttgagtggatgggaagaatcactcccagtgatggtaccacaacctacgcacagaagtttcagggcagagtcaccatgaccagggacccgtccacgaatactgtctacatagaactgaggagattgaaatcagaggacacggccgtatattattgtgtggcttacgacagagtaaccacatcggctggtacaggtgcctctgatatctggggccaagggacaatggtcaccgtctcttca

SEQ ID NO: 229 - DNA, 336 bp, Synthetic construct
  source 1..336: mol_type = other DNA
gatattgtgatgactcagtctccactctccctgcccgtcacccctggagagccggcctccatctcctgtaggtctagtcagagcctcctgcatggtgatggatacaactatttggattggtacctgcagaagccagggcggtctccacagctcctgatctatctgggttctcatcgggcctccggggtccctgacaggttcagtggcagtggatcaggcacagattttacactgagaatcagcagagtggaggctgaggatgttggaatttattactgcatgcaaggtctacaaactccgttcactttcggccctgggaccaaagtggatatcaaa

SEQ ID NO: 230 - DNA, 375 bp, Synthetic construct
  source 1..375: mol_type = other DNA
gaggtgcaagtggtggagtctgggggcggcttggtccagccgggggggtcgctgagactctcatgtgcagcctcaagtttcagcgtcactggcagttacatgacctgggtccgccaggctccagggaaggggctggagtcggtctcgctgatttatagtactgggagcacatactacgcagattccgtgaagggcagattcgtcatctccagagacgactccaaaaacatcttgtttctgcaaatgaacaacctgagagtcgaggacacgggtgtgtatttctgtgcgagacttgggcccgctggcggctcctggtcttgggagttctacggtctggacgtctggggccaggggaccacggtcaccgtcttctca

SEQ ID NO: 231 - DNA, 321 bp, Synthetic construct
  source 1..321: mol_type = other DNA
tgtgtccagatgacccagtctccatcattcctgtctgcatctgtaggagacagagtcaccatcagttgccgggccagtcagggcactaccagctatttagcctggtatcagcaaaaaccagggaaagcccccaagctcctgatctatggtgtgtccactttgcaaactggggtcccttcaaggttcagcggcagtggatctgggaccgacttcactctcacaatcagcaacctgcagcctgaagattttgcaacttattactgtcaacaggttaatattttcccatacactttcggccccggaaccaaggtggaaatcaaa

SEQ ID NO: 232 - DNA, 372 bp, Synthetic construct
  source 1..372: mol_type = other DNA
caggtgcaactggcgcagtctggggctgaggtgaggaggcctgggacctcagtgaaggtttcctgcaggtcatctgcatacgacttcatcgatgactccatacactgggtgcggcaggcccctggacaagggcttgagtggatggggaggatcgaccccagtggcgataccacaacctacgcaccgcagttccaggtcaggatcaccctgacccgggacacgtccacgagcacggcgtccatggagttgaacaggctcacatctcaagacacggccatgtattattgtgtggcttacgaaagagcaaccactttggctggtgtgggtgcctctgacgtctggggccaggggacatgggtcaccgtctcttca

SEQ ID NO: 233 - DNA, 336 bp, Synthetic construct
  source 1..336: mol_type = other DNA
gatattgtgatgactcagtctccactctccctgtccgtcacccctggagagccggcctccatctcctgcaggtctagtcagagcctcctgtatagagatggatacaactatttggattggtatctgcagaagccagggcagtctccacagctcctactctatttcgcttcttatcgggcctccggggtccctgacaggttcagtggcagtggatcaggcacagattttacactgaccatcaccagagtggagcctgaggatgttgggatttattactgcatgcagtctctacaaactccgttcactttcggccctgggaccaaactggatttcaaa

SEQ ID NO: 234 - DNA, 375 bp, Synthetic construct
  source 1..375: mol_type = other DNA
caggtgcagctacagcaatggggcgcaggactgttgaggccttcggagaccctgtccctcacctgcgctgtcagcggtgtgtccctcagtggggactacttgacctggatccgccagaccccagggaaggggctggagtggattggggaaattaatcatagtggaagcaccaactacaatccgtccctcaagagtcgagtcaccatatcagtagaaacgtccaagaaccacttctctctgaagatgaggtctgtgaccgccgcggactcggccctatattactgtgcgagaggctgggaatattgtcatgggactacctgctactcgaaggcttttgatatctggggccaagggacactggtcaccgtctcttca

SEQ ID NO: 235 - DNA, 321 bp, Synthetic construct
  source 1..321: mol_type = other DNA
gacatccagatgacccagtctccatcctccctgtctgcatctgtaggagacagggtcaccatcacttgccaggcgagtcaggacattagcaactatttaatttggtatcagcagaagccagggagagcccctaagctcctgatcttcgatgcatccaaattggaaaaaggggtcccaccaagattcagtggaagtggatctgggacatattttactttcaccatcagcagcctgcagcctgaagattttgcaacatattactgtcaacaatttcataatctcccagtcactttcggcggagggaccaaactggagaccaaa

SEQ ID NO: 236 - DNA, 369 bp, Synthetic construct
  source 1..369: mol_type = other DNA
gaggagcagctggtggagtccgggggaggcttggtccagcctggggggtccctgaaactctcctgtgctgcctctgggttcatcctcagtgactctactgttcactgggtccgccaggcttccgggagagggctggagtgggttggccgtattgctaacggttatgcgacatcatatgctgcgtcggtgaaaggcaggttcaccatctccacagatgattcagggaatacggcatatctggaaatgaacagcctgaaaaccgaggacacggccgtctattattgtactagccgaagtgtggtggtgactgatgtgggggccggtagggatgactactggggccagggaaccctggtcaccgtctcctca

SEQ ID NO: 237 - DNA, 336 bp, Synthetic construct
  source 1..336: mol_type = other DNA
gatatagtgatgactcagtctccactctccctgcccgtcacccctggagagccggcctccatctcctgcaggtctagtcagagcctcctacataggaatggatacaactatttggattggtacctacagaagccagggcagtctccacagctcctgatctggttgggttccaatcgggcctccggggtccctgacaggttcagtggcagtggatcaggcacagattttacactgacaatcagcagagtggaggctgaggatgttggggtttattactgcatgcaagatctacaaactcctcccactttcggcggagggaccaaggtggagatcatg

SEQ ID NO: 238 - DNA, 390 bp, Synthetic construct
  source 1..390: mol_type = other DNA
cagatcaccttgaaggagtctggtcctacgctgctgaaacccacacagaccctcacgctgacctgcaccttctctgggttctcactcaccactacgggggtggctgtgggctgggtccgtcagcccccaggaaaggccctggagtggcttgcactcatttactgggatgatgataagcgctacagtccatctctgaagagtagagtcaccatcaccaaggacacctccaaaaaccaggtactccttgcaatgaccgacatggaccctgttgacacagccacatactattgtgcacacttcgactacggtgaccccgaggtggtggccttatttgagtactcttactacatggacgtctggggcaaagggatcacggtcaccgtctcctca

SEQ ID NO: 239 - DNA, 333 bp, Synthetic construct
  source 1..333: mol_type = other DNA
cagtctgtgctgactcagccaccctcagtgtctgggacccccgggcagagggtcaccatctcttgttctggaagcagctccaacatcggaagtaattatgtatactggtaccagcacctcccaggaacggcccccaaactcctcatctatactaacaatcggcggccctcgggggtacctgatcgattctctggctccaagtctggcacctctgcctccctggccgtcagtgggctccggtccgaggatgaggctgattatttctgtgcagtatgggatgacagtgtgggtggtcactgggtgttcggcggagggaccaagctgaccgtccta

SEQ ID NO: 240 - DNA, 378 bp, Synthetic construct
  source 1..378: mol_type = other DNA
caggtacaactggaggagtcggggggaggcgtggtccagcctgggacgtccctgagactctcctgttcatcctctggagtcacacgcaacacttatgccgtacactgggtccgccaagttccaggcaaggggctggagtggctggcagcaacttcttatgacggaacaagtaaatattatccagaaaacgggcacggccgagtcagcatctccaaagagtattctactaatatggtgtatctggaaatttacaacctgagacctgaagacacggccgtgtatttctgtgccaaaggcccccaggggatatatagttatattggctacttctactacatggacgtctggggcaaggggaccacggtgaccgtctcctca

SEQ ID NO: 241 - DNA, 330 bp, Synthetic construct
  source 1..330: mol_type = other DNA
cagtctgccctgactcagcctgcctccgtgtctgggtctcctggacagtcgatcaccctctcctgcactggatccagggatgacgttggtgattatgactatgtctcctggtatcaacatcacccaggcaaagccccccgactcattatttatgatgtcactagtcggccctcaggagtctctcctcgattctcgggctccaagtctggcaacacggcctccctgaccatctctggcctccaggctgacgacgaggctgattattactgcaactcatatacaagcagcaactctgtggtcttcggcggagggaccaaggtgaccgtcctc

SEQ ID NO: 242 - DNA, 372 bp, Synthetic construct
  source 1..372: mol_type = other DNA
caggagcgactggcgcagtctgggactgaggtgaagaagcctggggcctcagtgaaggtttcctgcagggcacttggatacaccttcagcgattactccatacactgggtgcggcaggcccctagacaagggcttgagtggatgggaaagatcaatactagtggcggtaccacaacctacgcgcagaagttccaggccagagtcactttgaccagcgacacgtccacgagcacagcctccatggagctgagcagcctcaaaattgaagacacggccgtgtattactgtgtggcttacgagagagcaaccactttggctggtgcgggtgcttctgatatctggggccaggggacattggtcaccgtctcttca

SEQ ID NO: 243 - DNA, 336 bp, Synthetic construct
  source 1..336: mol_type = other DNA
gatattgtgatgactcagtctccactctccctgcccgtcacccctggagagccggcctccatctcctgcaggtctagtcagagcctcctgcatagtgatggatacaactatttggattggtacctgcagaagccagggcagtctccacacctcctgatctatttgggttctaatcgggcctccggggtccctgacaggttcagtggcagtggatcaggcacagattttacactgaaaatcaccagagtggagcctgaggatgttggggtttattactgcatgcaatctctacaaactccgttcactttcggccctgggaccaaagtggatgtcaaa

SEQ ID NO: 244 - DNA, 372 bp, Synthetic construct
  source 1..372: mol_type = other DNA
caggagcagctggtgcagtccggggctgaggtgaagaggcctgggacctcagtgaaggtctcctgcaaggcgtctggatatgccttcaccgattattctatacactgggtgcgacaggcccctggagtgggactggaatggatgggaaaaatttaccctggcgatggtcacgcactgtacgcacagaacttccagggcagagtcaccctgaccagggacacgtccacggcctctgtctacatggagctgaggagcctgagatctcaggacacggccgtctattattgtgtggcttacgagagagcaaccacactggctggcgcgggtgcttctgatatctggggccaagggacaatggtcaccgtatcttca

SEQ ID NO: 245 - DNA, 336 bp, Synthetic construct
  source 1..336: mol_type = other DNA
gacattgtgatgactcagtctccactctccctgcccgtcacccctggagagccggcctccatctcctgcaggtctagtcagagcctcctgcaaagtgatggatacaactatatggattggtacctgcagaagccagggcggtcgccacagctcctaatctacttgggttctcatcgggcctccggggtccctgacaggttcagtggcagtggctcaggcacagattttacactgagaatcagcagagtgaaggctgaggatgttggaatttattactgtatgcaatctctacaatctccgttcactttcggccctgggaccaaagtggatatcaaa

SEQ ID NO: 246 - DNA, 372 bp, Synthetic construct
  source 1..372: mol_type = other DNA
caggaacagtcggtgcagtctgggcctgaggtgaagaagcctggggcctctgtgaaggtctcctgcagggcatcagagttcaccttctccaccgactttatacactgggtgcgacaagcccctggacagggacttgagtggatgggaagaatcactcccagtgatggtaccacaacatacgcaccgaagtttcagggcagagtcgccgtgaccagggacccgtccacgaaaaatgtctacatacagttgactagattgaagtcagaggacacggccgtatattattgtgtggcatacgacagagcgaccacttcggccggtgcaggtgccactgatatttggggccaagggacactggtcaccgtctcctca

SEQ ID NO: 247 - DNA, 336 bp, Synthetic construct
  source 1..336: mol_type = other DNA
gatattgtgatgactcagtctccactctccctgcccgtcacccctggagagccggcctccatctcctgcaggtctagtcagagcctcctccatggtgatggatacaactatttggattggtacctgcagaggccagggcggtctccacaactcctgatctatctgggttctcatcgggcctccggggtccctgacaggttcagtggcagtggatcaggcacagattttacactgagaatcagcagagtggaggctgaggatgttggaatttattactgcatgcaaggtctgcaaactccgttcactttcggccctgggaccaaagtggatatcaaa

SEQ ID NO: 248 - DNA, 375 bp, Synthetic construct
  source 1..375: mol_type = other DNA
caggtgcagctgcagcagtcgggcccaggtctggtgaagccttcggagaccctgtccctcgcctgctctgtgtctggtggctccatgagtgacttctattggagttggattcggcagtccccagggacgggactggagtggattggctatgtccatcacagtgggaaggtcaactacaacccctcactcaaggcccgagtcaccatgtcactggacacgtccaagtacctcctctccctgaacttggcctctatgaccgctgcagactcggccgtctattactgtgcggccacctcggctttcgttgacagtagttcctactcccctccttactttgacttctggggccagggaaccctgatcaccgtctcctca

SEQ ID NO: 249 - DNA, 321 bp, Synthetic construct
  source 1..321: mol_type = other DNA
gacatccagctgacccagtctccatcctccctgtctgcatctgtaggagacagagtcaccattacttgccaggcgagtcacgacattaccaactatttaaattggtatcagcagacaccagggaaagcccctaggctcctgatctatgttgcgaccaatttggagacaggggtcccatcaagattcagtgggagtggatctgggacacattttactttaaccatcagcagcctgcagcctgaagatagtgcgacatattactgtcaacagtatgacaatctcccgatcactttcggcggagggaccagggtggagatcaga

SEQ ID NO: 250 - protein, 574 aa, Synthetic construct
MELLILKANAITTILTAVTFCFASGQNITEEFYQSTCSAVSKGYLSALRTGWYTSVITIELSNIKENKCNGTDAKVKLIKQELDKYKNAVTELQLLMQSTPPTNNRARRELPRFMNYTLNNAKKTNVTLSKKRKRRFLGFLLGVGSAIASGVAVSKVLHLEGEVNKIKSALLSTNKAVVSLSNGVSVLTFKVLDLKNYIDKQLLPILNKQSCSISNIETVIEFQQKNNRLLEITREFSVNAGVTTPVSTYMLTNSELLSLINDMPITNDQKKLMSNNVQIVRQQSYSIMSIIKEEVLAYVVQLPLYGVIDTPCWKLHTSPLCTTNTKEGSNICLTRTDRGWYCDNAGSVSFFPQAETCKVQSNRVFCDTMNSLTLPSEINLCNVDIFNPKYDCKIMTSKTDVCSSVITSLGAIVSCYGKCKCTASNKNRGIIKTFSNGCDYVSNKGMDTVSVGNTLYYVNKQEGKSLYVKGEPIINFYDPLVFPSDEFDASISQVNEKINQSLAFIRKSDELLHNVNAGKSTTNIMITTIIIVIIVILLSLIAVGLLLYCKARSTPVTLSKDQLSGINNIAFSN